European Patent Application EP 4 194 538 A1, published June 14, 2023. Title: DNA extraction vessel and Method for extracting DNA. Applicant: Go!Foton, Inc. Fukuzawa, Takashi. The sequence listing filed with the application follows.

SEQUENCE LISTING (9 sequences)

SEQ ID NO: 1 - DNA, 21 bp, Artificial Sequence
  Oncorhynchus mykiss forward PCR primer
agtctctccctgtatatcgtc

SEQ ID NO: 2 - DNA, 27 bp, Artificial Sequence
  Oncorhynchus mykiss reverse PCR primer
gatttagttcatgaagttgcgagagta

SEQ ID NO: 3 - DNA, 20 bp, Artificial Sequence
  Oncorhynchus mykiss probe
ccaacaactctttaaccatc

SEQ ID NO: 4 - DNA, 23 bp, Artificial Sequence
  Cyprinus carpio forward PCR primer
ggtgggttctcagtagacaatgc

SEQ ID NO: 5 - DNA, 22 bp, Artificial Sequence
  Cyprinus carpio reverse PCR primer
ggcggcaataacaaatggtagt

SEQ ID NO: 6 - DNA, 30 bp, Artificial Sequence
  Cyprinus carpio probe
cactaacacgattcttcgcattccacttcc

SEQ ID NO: 7 - DNA, 22 bp, Artificial Sequence
  Katsuwonus pelamis forward PCR primer
tacccctgacgtagaatcagcc

SEQ ID NO: 8 - DNA, 23 bp, Artificial Sequence
  Katsuwonus pelamis reverse PCR primer
ggccaatatgggagtaaatgcag

SEQ ID NO: 9 - DNA, 20 bp, Artificial Sequence
  Katsuwonus pelamis probe
tgccgagacgtaaacttcgg